European Patent Specification EP 4 211 260 B1, published April 9, 2025. Title: Application of Immobilized Enzymes for Nanopore Library Construction. Applicant: New England Biolabs, Inc. The sequence listing filed with the application follows.

SEQUENCE LISTING (3 sequences)

SEQ ID NO: 1 - DNA, 49 bp, Artificial Sequence
  Synthetic construct
  misc_feature: Gene32FAM-fw
  misc_feature (2)..(2): 6-FAMN
catggtgattacgattcttgcccagtatgtcaatacatcagtaaaaata

SEQ ID NO: 2 - DNA, 48 bp, Artificial Sequence
  Synthetic construct
  misc_feature: Gene32-rv
  misc_feature (1)..(1): p 5Phos
atttttactgatgtattgacatactgggcaagaatcgtaatcaccatg

SEQ ID NO: 3 - DNA, 64 bp, Artificial Sequence
  Synthetic construct
  misc_feature (1)..(1): p 5Phos
  misc_feature (32)..(32): ideoxyu
gatcggaagagcacacgtctgaactccagtcacactctttccctacacgacgctcttccgatct